European Patent Specification EP 4 062 974 B1, published May 8, 2024. Title: PHARMACEUTICAL COMPOSITION FOR PREVENTING OR TREATING CANCER. Applicant: L-Base Co., Ltd. The sequence listing filed with the application follows.

SEQUENCE LISTING (6 sequences)

SEQ ID NO: 1 - protein, 8 aa, Artificial Sequence
  Oligopeptide AQTGTGKT
AQTGTGKT

SEQ ID NO: 2 - protein, 2 aa, Artificial Sequence
  TG
TG

SEQ ID NO: 3 - protein, 2 aa, Artificial Sequence
  KT
KT

SEQ ID NO: 4 - protein, 4 aa, Artificial Sequence
  TGKT
TGKT

SEQ ID NO: 5 - protein, 6 aa, Artificial Sequence
  TGTGKT
TGTGKT

SEQ ID NO: 6 - protein, 7 aa, Artificial Sequence
  QTGTGKT
QTGTGKT